European Patent Specification EP 3 592 769 B1, published May 8, 2024. Title: Antibodies against PD-L1. Applicant: Genmab A/S. The sequence listing filed with the application follows.

SEQUENCE LISTING (115 sequences)

SEQ ID NO: 1 - protein, 119 aa, Homo Sapiens
EVQVVESGGGLVQPGGSLRLSCAASGFTFSRFWMSWVRQAPGKGLEWVANIKQDGGEKYYVDSVKGRFTISRDNAKNSLYLQMNSLRGEDTAVYYCARDDNWNGHFDYWGQGTLVTVSS

SEQ ID NO: 2 - protein, 8 aa, Homo Sapiens
GFTFSRFW

SEQ ID NO: 3 - protein, 8 aa, Homo Sapiens
IKQDGGEK

SEQ ID NO: 4 - protein, 12 aa, Homo Sapiens
ARDDNWNGHFDY

SEQ ID NO: 5 - protein, 107 aa, Homo Sapiens
DIQMTQSPSTLSASVGDRVTITCRASQSISSWLAWYQQKPGKAPNLLIYKASSLESGVPSRFSGSGSGTEFTLTISSLQPDDFATYYCQQYYGSYITFGQGTRLEIK

SEQ ID NO: 6 - protein, 6 aa, Homo Sapiens
QSISSW

SEQ ID NO: 7 - protein, 9 aa, Homo Sapiens
QQYYGSYIT

SEQ ID NO: 8 - protein, 121 aa, Homo Sapiens
QVQLVQSGSELKKPGASVMVSCKASGYTFTSYVMNWVRQAPGQGLEWMGWINSYTGNPTSAQGFTGRFVFSFDTSVNTAYLQISSLKAEDTAVYYCARGYCTSTSCYLDYWGQGTLVTVSS

SEQ ID NO: 9 - protein, 8 aa, Homo Sapiens
GYTFTSYV

SEQ ID NO: 10 - protein, 8 aa, Homo Sapiens
INSYTGNP

SEQ ID NO: 11 - protein, 14 aa, Homo Sapiens
ARGYCTSTSCYLDY

SEQ ID NO: 12 - protein, 108 aa, Homo Sapiens
SYELTQPPSVSVSPGHTARITCSGDALPKKYACWFQQKSGQAPVLVIYEDSKRPSGIPERFSGSTSGTMATLTISGAQVEDETDYYCYSADTSGTHRVFGGGTKLTVL

SEQ ID NO: 13 - protein, 6 aa, Homo Sapiens
ALPKKY

SEQ ID NO: 14 - protein, 11 aa, Homo Sapiens
YSADTSGTHRV

SEQ ID NO: 15 - protein, 108 aa, Artificial Sequence
  N/A
SYELTQPPSVSVSPGHTARITCSGDALPKKYASWFQQKSGQAPVLVIYEDSKRPSGIPERFSGSTSGTMATLTISGAQVEDETDYYCYSADTSGTHRVFGGGTKLTVL

SEQ ID NO: 16 - protein, 6 aa, Homo Sapiens
ALPKKY

SEQ ID NO: 17 - protein, 11 aa, Homo Sapiens
YSADTSGTHRV

SEQ ID NO: 18 - protein, 121 aa, Homo Sapiens
EVQLLEPGGGLVQPGGSLRLSCEASGSTFSTYAMSWVRQAPGKGLEWVSGFSGSGGFTFYADSVRGRFTISRDSSKNTLFLQMSSLRAEDTAVYYCAIPARGYNYGSFQHWGQGTLVTVSS

SEQ ID NO: 19 - protein, 8 aa, Homo Sapiens
GSTFSTYA

SEQ ID NO: 20 - protein, 8 aa, Homo Sapiens
FSGSGGFT

SEQ ID NO: 21 - protein, 14 aa, Homo Sapiens
AIPARGYNYGSFQH

SEQ ID NO: 22 - protein, 108 aa, Homo Sapiens
SYVLTQPPSVSVAPGQTARITCGGNNIGSKSVHWYQQKPGQAPVLVVYDDNDRPSGLPERFSGSNSGNTATLTISRVEAGDEADYYCQVWDSSSDHVVFGGGTKLTVL

SEQ ID NO: 23 - protein, 6 aa, Homo Sapiens
NIGSKS

SEQ ID NO: 24 - protein, 11 aa, Homo Sapiens
QVWDSSSDHVV

SEQ ID NO: 25 - protein, 125 aa, Homo Sapiens
EVKLVESGGGLVQPGGSLRLSCAASGFTFNTYAMNWVRQAPGKGLEWVARIRSKYNNYATYYADSVKDRFTISRDDSKSSLYLQMNNLKTEDTAMYYCVRHGNFGNSYVSWFAYWGQGTLVTVSS

SEQ ID NO: 26 - protein, 8 aa, Homo Sapiens
GFTFNTYA

SEQ ID NO: 27 - protein, 10 aa, Homo Sapiens
IRSKYNNYAT

SEQ ID NO: 28 - protein, 16 aa, Homo Sapiens
VRHGNFGNSYVSWFAY

SEQ ID NO: 29 - protein, 109 aa, Homo Sapiens
QAVVTQEPSFSVSPGGTVTLTCRSSTGAVTTSNYANWVQQTPGQAFRGLIGGTNKRAPGVPARFSGSLIGDKAALTITGAQADDESIYFCALWYSNLWVFGGGTKLTVL

SEQ ID NO: 30 - protein, 9 aa, Homo Sapiens
TGAVTTSNY

SEQ ID NO: 31 - protein, 9 aa, Homo Sapiens
ALWYSNLWV

SEQ ID NO: 32 - protein, 123 aa, Homo Sapiens
EVQLVESGGGLVQPGGSLRLSCAASGFTFSSYWMSWVRQAPGKGLEWVANIKQDGNEKYYVDSVKGRFTISRDNAKNSLYVQMNSLRAEDTAVYYCARDLYYGSGTYPPFDYWGQGTLVTVSS

SEQ ID NO: 33 - protein, 8 aa, Homo Sapiens
GFTFSSYW

SEQ ID NO: 34 - protein, 8 aa, Homo Sapiens
IKQDGNEK

SEQ ID NO: 35 - protein, 16 aa, Homo Sapiens
ARDLYYGSGTYPPFDY

SEQ ID NO: 36 - protein, 107 aa, Homo Sapiens
DIQMTQSPSTLSASVGDRVTITCRASQSISSWLAWYLQKPGKAPKLLIYKASSLESGVPSRFSGSGSGTEFTLTISSLQPDDFATYYCQQYHSSSYTFGQGTKLEIK

SEQ ID NO: 37 - protein, 6 aa, Homo Sapiens
QSISSW

SEQ ID NO: 38 - protein, 9 aa, Homo Sapiens
QQYHSSSYT

SEQ ID NO: 39 - protein, 125 aa, Artificial Sequence
  N/A
EVKLVESGGGLVQPGGSLRLSCAASGFTFNPYAMNWVRQAPGKGLEWVARIRSKYNNYATYYADSVKDRFTISRDDSKSSLYLQMNNLKTEDTAMYYCVRHGNFGNSYVSWFAYWGQGTLVTVSS

SEQ ID NO: 40 - protein, 125 aa, Artifical Sequence
EVKLVESGGGLVQPGGSLRLSCAASGFTFNMYAMNWVRQAPGKGLEWVARIRSKYNNYATYYADSVKDRFTISRDDSKSSLYLQMNNLKTEDTAMYYCVRHGNFGNSYVSWFAYWGQGTLVTVSS

SEQ ID NO: 41 - protein, 126 aa, Artificial Sequence
  N/A
EVKLVESGGGLVQPGGSLRLSCAASGFTFNTYAMNWVRQAPGKGLEWVARIRSKYNNYATYYADSVKDRFTISRDDSKSSLYLQMNNLKTEDTAMYYCVRHGNFGNSYVSWFAYVWGQGTLVTVSS

SEQ ID NO: 42 - protein, 125 aa, Artificial Sequence
  N/A
EVKLVESGGGLVQPGGSLRLSCAASGFTFNTYAMNWVRQAPGKGLEWVARIRSKYNNYATYYADSVKDRFTISRDDSKSSLYLQMNNLKTEDTAMYYCVRHGNFGNSYVSWFAMWGQGTLVTVSS

SEQ ID NO: 43 - protein, 125 aa, Artificial Sequence
  N/A
EVKLVESGGGLVQPGGSLRLSCAASGFTFNTYAMNWVRQAPGKGLEWVARIRSKYNNYATYYADSVKDRFTISRDDSKSSLYLQMNNLKTEDTAMYYCVRHGNFGNSYVSWFARWGQGTLVTVSS

SEQ ID NO: 44 - protein, 125 aa, Artificial Sequence
  N/A
EVKLVESGGGLVQPGGSLRLSCAASGFTFNTYAMNWVRQAPGKGLEWVARIRSKYNNYATYYADSVKDRFTISRDDSKSSLYLQMNNLKTEDTAMYYCVRHGNFGNSYVAWFAYWGQGTLVTVSS

SEQ ID NO: 45 - protein, 125 aa, Artificial Sequence
  N/A
EVKLVESGGGLVQPGGSLRLSCAASGFTFNTYAMNWVRQAPGKGLEWVARIRSKYNNYATYYADSVKDRFTISRDDSKSSLYLQMNNLKTEDTAMYYCVRGGNFGNSYVSWFAYWGQGTLVTVSS

SEQ ID NO: 46 - protein, 121 aa, Homo Sapiens
EVQLVESGGGLVQPGRSLRLSCAASGFTFDDYAMHWVRQGPGKGLEWVSGIRWNSGSMHYADSVKGRFTISRDNAKSSLYLQMNSLRAEDTALYYCARAPWYSGAWHPDYWGQGTLVTVSS

SEQ ID NO: 47 - protein, 8 aa, Homo Sapiens
GFTFDDYA

SEQ ID NO: 48 - protein, 8 aa, Homo Sapiens
IRWNSGSM

SEQ ID NO: 49 - protein, 14 aa, Homo Sapiens
ARAPWYSGAWHPDY

SEQ ID NO: 50 - protein, 110 aa, Artificial Sequence
  N/A
QSALTQPRSVSGSPGQSVTISCTGTSSDVGTYNYVSWYQQHPGKAPKLMIYDVIKRPSGVPDRFSGSKSGNTASLTLSGLQAEDEADYYCSSYAGTYTLLFGGGTKLTVL

SEQ ID NO: 51 - protein, 9 aa, Homo Sapiens
SSDVGTYNY

SEQ ID NO: 52 - protein, 10 aa, Artificial Sequence
  N/A
SSYAGTYTLL

SEQ ID NO: 53 - protein, 127 aa, Artificial Sequence
  N/A
EVQMLESGGGLVQPGGSLRLSCAASGFTFRSYAMSWVRQAPGKGLEWVSGIGDSGGSTYHADSVKGRFTISRDNSKNTLYLQMNSLRAEDTAVYYCAKLGQSSGWYDHYYYYGMDVWGQGTTVTVSS

SEQ ID NO: 54 - protein, 8 aa, Homo Sapiens
GFTFRSYA

SEQ ID NO: 55 - protein, 8 aa, Homo Sapiens
IGDSGGST

SEQ ID NO: 56 - protein, 20 aa, Artificial Sequence
  N/A
AKLGQSSGWYDHYYYYGMDV

SEQ ID NO: 57 - protein, 106 aa, Artificial Sequence
  N/A
SYELTQPPSVSVSPGQTASITCSGDKLGNKYVSWFQQKPGQSPVLVIYRDSERPSGIPERFSGSNSGNTATLTISGTQAVDEADFYCQAWDSSTVVFGGGTKLTVL

SEQ ID NO: 58 - protein, 6 aa, Homo Sapiens
KLGNKY

SEQ ID NO: 59 - protein, 9 aa, Homo Sapiens
QAWDSSTVV

SEQ ID NO: 60 - protein, 120 aa, Homo Sapiens
QVQLQESGPGLVKPSDTLSLTCAVSDYSISSNDWWGWIRQPPGKGLEWIGYIYYSGTGYYNPSLKSRVTISIDTSKNQFSLKLNSVTAVDTAVYYCARTRVGARRAFDYWGQGTLVTVSS

SEQ ID NO: 61 - protein, 9 aa, Homo Sapiens
DYSISSNDW

SEQ ID NO: 62 - protein, 7 aa, Homo Sapiens
IYYSGTG

SEQ ID NO: 63 - protein, 13 aa, Homo Sapiens
ARTRVGARRAFDY

SEQ ID NO: 64 - protein, 108 aa, Homo Sapiens
SYVLTQPPSVSVAPGQTARITCGGNNIGSKSVHWYQQKPGQAPVLVVYDDSDRPSGIPERFSGSNSGNTATLTISRVEAGDEADYYCQVWDSSSDHVVFGGGTKLTVL

SEQ ID NO: 65 - protein, 6 aa, Homo Sapiens
NIGSKS

SEQ ID NO: 66 - protein, 11 aa, Homo Sapiens
QVWDSSSDHVV

SEQ ID NO: 67 - protein, 123 aa, Homo Sapiens
QVQLVESGGGLVKPGGSLRLSCAASGFTFSDYYMSWIRQAPGKGLEWVSYIGSSSNTIYYADSVKGRFTISRDNAKNSLYLQMNSLRAEDTAVYSCARDRVKYGSPGSLFDYWGQGTLVTVSS

SEQ ID NO: 68 - protein, 8 aa, Homo Sapiens
GFTFSDYY

SEQ ID NO: 69 - protein, 8 aa, Homo Sapiens
IGSSSNTI

SEQ ID NO: 70 - protein, 16 aa, Homo Sapiens
ARDRVKYGSPGSLFDY

SEQ ID NO: 71 - protein, 108 aa, Homo Sapiens
SYELTQPPSVSVSPGQTARITCSGDALPKKYAFWYQQKSGQAPVLVIYEDSKRPSGIPERFSGSSSGTMATLTISGAQVEDEADYYCYSTASSGDHRVFGGGTKLTVL

SEQ ID NO: 72 - protein, 6 aa, Homo Sapiens
ALPKKY

SEQ ID NO: 73 - protein, 11 aa, Homo Sapiens
YSTASSGDHRV

SEQ ID NO: 74 - protein, 118 aa, Homo Sapiens
EVQLVESGGGLVQPGGSLRLSCAASGFTFSDSWIHWYRQAPGKGLEWYAWISPYGGSTYYADSVKGRFTISADTSKNTAYLQMNSLRAEDTAVYYCARRHWPGGFDYWGQGTLVTVSS

SEQ ID NO: 75 - protein, 8 aa, Homo Sapiens
GFTFSDSW

SEQ ID NO: 76 - protein, 8 aa, Homo Sapiens
ISPYGGST

SEQ ID NO: 77 - protein, 11 aa, Homo Sapiens
ARRHWPGGFDY

SEQ ID NO: 78 - protein, 107 aa, Homo Sapiens [sequence omitted]

SEQ ID NO: 79 - protein, 6 aa, Homo Sapiens
QDVSTA

SEQ ID NO: 80 - protein, 9 aa, Homo Sapiens
QQYLYHPAT

SEQ ID NO: 81 - protein, 121 aa, Homo Sapiens
EVQLVESGGGLVQPGGSLRLSCAASGFTFSRYWMSWVRQAPGKGLEWVANIKQDGSEKYYVDSVKGRFTISRDNAKNSLYLQMNSLRAEDTAVYYCAREGGWFGELAFDYWGQGTLVTVSS

SEQ ID NO: 82 - protein, 8 aa, Homo Sapiens
GFTFSRYW

SEQ ID NO: 83 - protein, 8 aa, Homo Sapiens
IKQDGSEK

SEQ ID NO: 84 - protein, 14 aa, Homo Sapiens
AREGGWFGELAFDY

SEQ ID NO: 85 - protein, 108 aa, Homo Sapiens
EIVLTQSPGTLSLSPGERATLSCRASQRVSSSYLAWYQQKPGQAPRLLIYDASSRATGIPDRFSGSGSGTDFTLTISRLEPEDFAVYYCQQYGSLPWTFGQGTKVEIK

SEQ ID NO: 86 - protein, 7 aa, Homo Sapiens
QRVSSSY

SEQ ID NO: 87 - protein, 3 aa, Homo Sapiens
DAS

SEQ ID NO: 88 - protein, 9 aa, Homo Sapiens
QQYGSLPWT

SEQ ID NO: 89 - protein, 330 aa, Artificial Sequence
  N/A
ASTKGPSVFPLAPSSKSTSGGTAALGCLVKDYFPEPVTVSWNSGALTSGVHTFPAVLQSSGLYSLSSVVTVPSSSLGTQTYICNVNHKPSNTKVDKRVEPKSCDKTHTCPPCPAPEFEGGPSVFLFPPKPKDTLMISRTPEVTCVVVAVSHEDPEVKFNWYVDGVEVHNAKTKPREEQYNSTYRVVSVLTVLHQDWLNGKEYKCKVSNKALPAPIEKTISKAKGQPREPQVYTLPPSREEMTKNQVSLTCLVKGFYPSDIAVEWESNGQPENNYKTTPPVLDSDGSFFLYSRLTVDKSRWQQGNVFSCSVMHEALHNHYTQKSLSLSPGK

SEQ ID NO: 90 - protein, 330 aa, Artificial Sequence
  N/A
ASTKGPSVFPLAPSSKSTSGGTAALGCLVKDYFPEPVTVSWNSGALTSGVHTFPAVLQSSGLYSLSSVVTVPSSSLGTQTYICNVNHKPSNTKVDKRVEPKSCDKTHTCPPCPAPEFEGGPSVFLFPPKPKDTLMISRTPEVTCVVVAVSHEDPEVKFNWYVDGVEVHNAKTKPREEQYNSTYRVVSVLTVLHQDWLNGKEYKCKVSNKALPAPIEKTISKAKGQPREPQVYTLPPSREEMTKNQVSLTCLVKGFYPSDIAVEWESNGQPENNYKTTPPVLDSDGSFLLYSKLTVDKSRWQQGNVFSCSVMHEALHNHYTQKSLSLSPGK

SEQ ID NO: 91 - protein, 107 aa, Homo Sapiens [sequence omitted]

SEQ ID NO: 92 - protein, 106 aa, Homo Sapiens
GQPKAAPSVTLFPPSSEELQANKATLVCLISDFYPGAVTVAWKADSSPVKAGVETTTPSKQSNNKYAASSYLSLTPEQWKSHRSYSCQVTHEGSTVEKTVAPTECS

SEQ ID NO: 93 - protein, 330 aa, Homo Sapiens
ASTKGPSVFPLAPSSKSTSGGTAALGCLVKDYFPEPVTVSWNSGALTSGVHTFPAVLQSSGLYSLSSVVTVPSSSLGTQTYICNVNHKPSNTKVDKRVEPKSCDKTHTCPPCPAPELLGGPSVFLFPPKPKDTLMISRTPEVTCVVVDVSHEDPEVKFNWYVDGVEVHNAKTKPREEQYNSTYRVVSVLTVLHQDWLNGKEYKCKVSNKALPAPIEKTISKAKGQPREPQVYTLPPSREEMTKNQVSLTCLVKGFYPSDIAVEWESNGQPENNYKTTPPVLDSDGSFFLYSKLTVDKSRWQQGNVFSCSVMHEALHNHYTQKSLSLSPGK

SEQ ID NO: 94 - protein, 290 aa, Homo Sapiens
MRIFAVFIFMTYWHLLNAFTVTVPKDLYVVEYGSNMTIECKFPVEKQLDLAALIVYWEMEDKNIIQFVHGEEDLKVQHSSYRQRARLLKDQLSLGNAALQITDVKLQDAGVYRCMISYGGADYKRITVKVNAPYNKINQRILVVDPVTSEHELTCQAEGYPKAEVIWTSSDHQVLSGKTTTTNSKREEKLFNVTSTLRINTTTNEIFYCTFRRLDPEENHTAELVIPELPLAHPPNERTHLVILGAILLCLGVALTFIFRLRKGRMMDVKKCGIQDTNSKKQSDTHLEET

SEQ ID NO: 95 - protein, 186 aa, Homo Sapiens
QDGNEEMGGITQTPYKVSISGTTVILTCPQYPGSEILWQHNDKNIGGDEDDKNIGSDEDHLSLKEFSELEQSGYYVCYPRGSKPEDANFYLYLRARVCENCMEMDVMSVATIVIVDICITGGLLLLVYYWSKNRKAKAKPVTRGAGAGGRQRGQNKERPPPVPNPDYEPIRKGQRDLYSGLNQRRI

SEQ ID NO: 96 - protein, 107 aa, Homo Sapiens
GQPREPQVYTLPPSRDELTKNQVSLTCLVKGFYPSDIAVEWESNGQPENNYKTTPPVLDSDGSFFLYSKLTVDKSRWQQGNVFSCSVMHEALHNHYTQKSLSLSPGK

SEQ ID NO: 97 - protein, 107 aa, Homo Sapiens
GQPREPQVYTLPPSREEMTKNQVSLTCLVKGFYPSDIAVEWESNGQPENNYKTTPPVLDSDGSFFLYSKLTVDKSRWQQGNVFSCSVMHEALHNHYTQKSLSLSPGK

SEQ ID NO: 98 - protein, 107 aa, Homo Sapiens
GQPREPQVYTLPPSRDELTKNQVSLTCLVKGFYPSDIAVEWESNGQPENNYKTTPPVLDSDGSFFLYSKLTVDKSRWQQGNVFSCSVMHEGLHNHYTQKSLSLSPGK

SEQ ID NO: 99 - protein, 8 aa, Artificial Sequence
  N/A
GFTFNPYA

SEQ ID NO: 100 - protein, 8 aa, Artificial Sequence
  N/A
GFTFNMYA

SEQ ID NO: 101 - protein, 16 aa, Artificial Sequence
  N/A
VRHGNFGNSYVSWFAV

SEQ ID NO: 102 - protein, 16 aa, Artificial Sequence
  N/A
VRHGNFGNSYVSWFAM

SEQ ID NO: 103 - protein, 16 aa, Artificial Sequence
  N/A
VRHGNFGNSYVSWFAR

SEQ ID NO: 104 - protein, 16 aa, Artificial Sequence
  N/A
VRHGNFGNSYVAWFAY

SEQ ID NO: 105 - protein, 16 aa, Artificial Sequence
  N/A
VRGGNFGNSYVSWFAY

SEQ ID NO: 106 - protein, 124 aa, Homo Sapiens
HMQLVESGGGVAQPGRSLRLSCAASGFTFSNYGMHWVRQAPGRGLEWLAVMSYDGETKYYADSVKGRFTISRDNSENTLFLQMNSLRAEDTAVYYCAKDTSNGWNYYFYGMDVWGQGTTVTVSS

SEQ ID NO: 107 - protein, 8 aa, Homo Sapiens
GFTFSNYG

SEQ ID NO: 108 - protein, 8 aa, Homo Sapiens
MSYDGETK

SEQ ID NO: 109 - protein, 17 aa, Homo Sapiens
AKDTSNGWNYYFYGMDV

SEQ ID NO: 110 - protein, 108 aa, Homo Sapiens
SYELTQPPSVSVSPGQTARITCSGDALPKKFASWYQQKSGQAPVLVIYEDSKRPSGIPERVSGSSSGTMATLTISGAQTEDEADYYCYSTDRSGYHWVFGGGTKLTVL

SEQ ID NO: 111 - protein, 6 aa, Homo Sapiens
ALPKKF

SEQ ID NO: 112 - protein, 11 aa, Homo Sapiens
YSTDRSGYHWV

SEQ ID NO: 113 - protein, 330 aa, Homo Sapiens; identical to SEQ ID NO: 93

SEQ ID NO: 114 - protein, 330 aa, Artificial Sequence
  N/A
ASTKGPSVFPLAPSSKSTSGGTAALGCLVKDYFPEPVTVSWNSGALTSGVHTFPAVLQSSGLYSLSSVVTVPSSSLGTQTYICNVNHKPSNTKVDKRVEPKSCDKTHTCPPCPAPELLGGPSVFLFPPKPKDTLMISRTPEVTCVVVDVSHEDPEVKFNWYVDGVEVHNAKTKPREEQYNSTYRVVSVLTVLHQDWLNGKEYKCKVSNKALPAPIEKTISKAKGQPREPQVYTLPPSREEMTKNQVSLTCLVKGFYPSDIAVEWESNGQPENNYKTTPPVLDSDGSFFLYSRLTVDKSRWQQGNVFSCSVMHEALHNHYTQKSLSLSPGK

SEQ ID NO: 115 - protein, 330 aa, Artificial Sequence
  N/A
ASTKGPSVFPLAPSSKSTSGGTAALGCLVKDYFPEPVTVSWNSGALTSGVHTFPAVLQSSGLYSLSSVVTVPSSSLGTQTYICNVNHKPSNTKVDKRVEPKSCDKTHTCPPCPAPELLGGPSVFLFPPKPKDTLMISRTPEVTCVVVDVSHEDPEVKFNWYVDGVEVHNAKTKPREEQYNSTYRVVSVLTVLHQDWLNGKEYKCKVSNKALPAPIEKTISKAKGQPREPQVYTLPPSREEMTKNQVSLTCLVKGFYPSDIAVEWESNGQPENNYKTTPPVLDSDGSFLLYSKLTVDKSRWQQGNVFSCSVMHEALHNHYTQKSLSLSPGK